European Patent Application EP 4 722 227 A1, published April 8, 2026. Title: Complexes, pharmaceutical compositions, vaccines and their applications. Applicant: Enyu Pharma Co. The sequence listing filed with the application follows.

SEQUENCE LISTING (13 sequences)

SEQ ID NO: 1 - protein, 18 aa, synthetic construct
  CARBOHYD 10: note = O-linked glycosylation
QVSPFGEVFNATRFASVC

SEQ ID NO: 2 - protein, 18 aa, synthetic construct
QVSPFGEVFNATRFASVC

SEQ ID NO: 3 - protein, 17 aa, synthetic construct
  CARBOHYD 8: note = O-linked glycosylation
  CARBOHYD 10: note = O-linked glycosylation
SNFRVQPTESIVRFNIC

SEQ ID NO: 4 - protein, 17 aa, synthetic construct
SNFRVQPTESIVRFNIC

SEQ ID NO: 5 - protein, 19 aa, synthetic construct
  CARBOHYD 8: note = O-linked glycosylation
GVTSAPDTRPAPGSTAPPA

SEQ ID NO: 6 - protein, 18 aa, synthetic construct
  CARBOHYD 9: note = O-linked glycosylation
  CARBOHYD 10: note = O-linked glycosylation
GFRRTTPPTTATPIRHRC

SEQ ID NO: 7 - protein, 18 aa, synthetic construct
GFRRTTPPTTATPIRHRC

SEQ ID NO: 8 - protein, 62 aa, synthetic construct
  CARBOHYD 10: note = O-linked glycosylation
  CARBOHYD 11: note = O-linked glycosylation
EVHISGLYPHEARGARGTHRTHRPROPROTHRTHRALATHRPROILEARGHISARGPROCYS

SEQ ID NO: 9 - protein, 20 aa, synthetic construct
  CARBOHYD 7: note = O-linked glycosylation
  CARBOHYD 10: note = O-linked glycosylation
  CARBOHYD 11: note = O-linked glycosylation
HGFRRTTPPTTATPIRHRPC

SEQ ID NO: 10 - protein, 20 aa, synthetic construct
  CARBOHYD 10: note = O-linked glycosylation
  CARBOHYD 11: note = O-linked glycosylation
HGFRRTTPPTTATPIRHRPC

SEQ ID NO: 11 - protein, 20 aa, synthetic construct
  CARBOHYD 7: note = O-linked glycosylation
  CARBOHYD 10: note = O-linked glycosylation
  CARBOHYD 11: note = O-linked glycosylation
HGFRRTTPPTTATPIRHRPC

SEQ ID NO: 12 - protein, 20 aa, synthetic construct
  CARBOHYD 10: note = O-linked glycosylation
  CARBOHYD 11: note = O-linked glycosylation
HGFRRTTPPTTATPIRHRPC

SEQ ID NO: 13 - protein, 20 aa, synthetic construct
HGFRRTTPPTTATPIRHRPC